European Patent Specification EP 4 021 487 B1, published December 27, 2023. Title: ANTIGENIC PEPTIDES FOR PREVENTION AND TREATMENT OF B-CELL MALIGNANCY. Applicant: ENTEROME SA. The sequence listing filed with the application follows.

SEQUENCE LISTING (509 sequences)

SEQ ID NO: 1 - protein, 9 aa, Artificial Sequence
  peptide
FLLFLTPIL

SEQ ID NO: 2 - protein, 9 aa, Artificial
  peptide
FLLFLTPLL

SEQ ID NO: 3 - protein, 9 aa, Artificial
  peptide
FMLFLTPRI

SEQ ID NO: 4 - protein, 9 aa, Artificial
  peptide
GLLFLTPLA

SEQ ID NO: 5 - protein, 9 aa, Artificial
  peptide
GLLFLTPLL

SEQ ID NO: 6 - protein, 9 aa, Artificial
  peptide
GLLFLTPLM

SEQ ID NO: 7 - protein, 9 aa, Artificial
  peptide
ILLFLTPLL

SEQ ID NO: 8 - protein, 9 aa, Artificial
  peptide
SLLFLTPLL

SEQ ID NO: 9 - protein, 9 aa, Artificial
  peptide
TLLFLTPLI

SEQ ID NO: 10 - protein, 9 aa, Artificial
  peptide
TLLFLTPML

SEQ ID NO: 11 - protein, 9 aa, Artificial
  peptide
VLLFLTPML

SEQ ID NO: 12 - protein, 9 aa, Artificial
  peptide
YLLFLTPVL

SEQ ID NO: 13 - protein, 9 aa, Artificial
  peptide
ALSLGLPGL

SEQ ID NO: 14 - protein, 9 aa, Artificial
  peptide
ALSLGLPLL

SEQ ID NO: 15 - protein, 9 aa, Artificial
  peptide
ALSLGLPML

SEQ ID NO: 16 - protein, 9 aa, Artificial
  peptide
ALSLGLPQL

SEQ ID NO: 17 - protein, 9 aa, Artificial
  peptide
ALSLGLPRL

SEQ ID NO: 18 - protein, 9 aa, Artificial
  peptide
AMSLGLPCL

SEQ ID NO: 19 - protein, 9 aa, Artificial
  peptide
AMSLGLPML

SEQ ID NO: 20 - protein, 9 aa, Artificial
  peptide
FLSLGLPIL

SEQ ID NO: 21 - protein, 9 aa, Artificial
  peptide
FLSLGLPKL

SEQ ID NO: 22 - protein, 9 aa, Artificial
  peptide
ILSLGLPIL

SEQ ID NO: 23 - protein, 9 aa, Artificial
  peptide
KLSLGLPVL

SEQ ID NO: 24 - protein, 9 aa, Artificial
  peptide
LLSLGLPFL

SEQ ID NO: 25 - protein, 9 aa, Artificial
  peptide
LLSLGLPGL

SEQ ID NO: 26 - protein, 9 aa, Artificial
  peptide
MLSLGLPIL

SEQ ID NO: 27 - protein, 9 aa, Artificial
  peptide
RLSLGLPGL

SEQ ID NO: 28 - protein, 9 aa, Artificial
  peptide
SLSLGLPIL

SEQ ID NO: 29 - protein, 9 aa, Artificial
  peptide
SLSLGLPKL

SEQ ID NO: 30 - protein, 9 aa, Artificial
  peptide
VLSLGLPLL

SEQ ID NO: 31 - protein, 9 aa, Artificial
  peptide
VLSLGLPTA

SEQ ID NO: 32 - protein, 9 aa, Artificial
  peptide
VLSLGLPTV

SEQ ID NO: 33 - protein, 9 aa, Artificial
  peptide
YLSLGLPIL

SEQ ID NO: 34 - protein, 9 aa, Artificial
  peptide
LLVGILHLV

SEQ ID NO: 35 - protein, 9 aa, Artificial
  peptide
SLVGILHII

SEQ ID NO: 36 - protein, 9 aa, Artificial
  peptide
FLAYLIFGL

SEQ ID NO: 37 - protein, 9 aa, Artificial
  peptide
FLAYLIFTL

SEQ ID NO: 38 - protein, 9 aa, Artificial
  peptide
RLAYLIFLL

SEQ ID NO: 39 - protein, 9 aa, Artificial
  peptide
YLAYLIFEL

SEQ ID NO: 40 - protein, 9 aa, Artificial
  peptide
LQMGGFYLL

SEQ ID NO: 41 - protein, 9 aa, Artificial
  peptide
AILGGLLLI

SEQ ID NO: 42 - protein, 9 aa, Artificial
  peptide
ALLGGLLLI

SEQ ID NO: 43 - protein, 9 aa, Artificial
  peptide
ALLGGLLML

SEQ ID NO: 44 - protein, 9 aa, Artificial
  peptide
FALGGLLTV

SEQ ID NO: 45 - protein, 9 aa, Artificial
  peptide
FLLGGLLLI

SEQ ID NO: 46 - protein, 9 aa, Artificial
  peptide
FLLGGLLMV

SEQ ID NO: 47 - protein, 9 aa, Artificial
  peptide
GMLGGLLLI

SEQ ID NO: 48 - protein, 9 aa, Artificial
  peptide
GMLGGLLML

SEQ ID NO: 49 - protein, 9 aa, Artificial
  peptide
HILGGLLMV

SEQ ID NO: 50 - protein, 9 aa, Artificial
  peptide
IILGGLLVV

SEQ ID NO: 51 - protein, 9 aa, Artificial
  peptide
ILLGGLLLI

SEQ ID NO: 52 - protein, 9 aa, Artificial
  peptide
LLLGGLLLI

SEQ ID NO: 53 - protein, 9 aa, Artificial
  peptide
LLLGGLLMI

SEQ ID NO: 54 - protein, 9 aa, Artificial
  peptide
NLLGGLLLI

SEQ ID NO: 55 - protein, 9 aa, Artificial
  peptide
SILGGLLLI

SEQ ID NO: 56 - protein, 9 aa, Artificial
  peptide
SLLGGLLLI

SEQ ID NO: 57 - protein, 9 aa, Artificial
  peptide
SLLGGLLML

SEQ ID NO: 58 - protein, 9 aa, Artificial
  peptide
SMLGGLLLI

SEQ ID NO: 59 - protein, 9 aa, Artificial
  peptide
TLLGGLLMI

SEQ ID NO: 60 - protein, 9 aa, Artificial
  peptide
YALGGLLEV

SEQ ID NO: 61 - protein, 9 aa, Artificial
  peptide
YILGGLLMV

SEQ ID NO: 62 - protein, 9 aa, Artificial
  peptide
YMLGGLLLI

SEQ ID NO: 63 - protein, 9 aa, Artificial
  peptide
YVLGGLLMI

SEQ ID NO: 64 - protein, 9 aa, Artificial
  peptide
YVLGGLLMV

SEQ ID NO: 65 - protein, 9 aa, Artificial
  peptide
AMNSLSLYI

SEQ ID NO: 66 - protein, 9 aa, Artificial
  peptide
ILNSLSLKI

SEQ ID NO: 67 - protein, 9 aa, Artificial
  peptide
ILNSLSLKL

SEQ ID NO: 68 - protein, 9 aa, Artificial
  peptide
ILNSLSLLL

SEQ ID NO: 69 - protein, 9 aa, Artificial
  Artificial
LLNSLSLFL

SEQ ID NO: 70 - protein, 9 aa, Artificial
  peptide
YMNSLSLAL

SEQ ID NO: 71 - protein, 9 aa, Artificial
  peptide
FLIPAGIFL

SEQ ID NO: 72 - protein, 9 aa, Artificial
  peptide
ILIPAGIYL

SEQ ID NO: 73 - protein, 9 aa, Artificial
  peptide
LLIPAGIAV

SEQ ID NO: 74 - protein, 9 aa, Artificial
  peptide
LLIPAGIEL

SEQ ID NO: 75 - protein, 9 aa, Artificial
  peptide
LLIPAGIGL

SEQ ID NO: 76 - protein, 9 aa, Artificial
  peptide
LLIPAGILI

SEQ ID NO: 77 - protein, 9 aa, Artificial
  peptide
LLIPAGILL

SEQ ID NO: 78 - protein, 9 aa, Artificial
  peptide
MLIPAGIPA

SEQ ID NO: 79 - protein, 9 aa, Artificial
  peptide
MMIPAGIAV

SEQ ID NO: 80 - protein, 9 aa, Artificial
  peptide
VMIPAGIFL

SEQ ID NO: 81 - protein, 9 aa, Artificial
  peptide
FLFLGILGL

SEQ ID NO: 82 - protein, 9 aa, Artificial
  peptide
FLFLGILPL

SEQ ID NO: 83 - protein, 9 aa, Artificial
  peptide
MLFLGILSV

SEQ ID NO: 84 - protein, 9 aa, Artificial
  peptide
YLFLGILGI

SEQ ID NO: 85 - protein, 9 aa, Artificial
  peptide
YLFLGILGL

SEQ ID NO: 86 - protein, 9 aa, Artificial
  peptide
YLFLGILSL

SEQ ID NO: 87 - protein, 9 aa, Artificial
  peptide
YLFLGILYL

SEQ ID NO: 88 - protein, 9 aa, Artificial
  peptide
FLSNDTVLL

SEQ ID NO: 89 - protein, 9 aa, Artificial
  peptide
FLSNDTVPL

SEQ ID NO: 90 - protein, 9 aa, Artificial
  peptide
FLSNDTVSA

SEQ ID NO: 91 - protein, 9 aa, Artificial
  peptide
FMSNDTVKV

SEQ ID NO: 92 - protein, 9 aa, Artificial
  peptide
ILSNDTVWL

SEQ ID NO: 93 - protein, 9 aa, Artificial
  peptide
KMSNDTVVL

SEQ ID NO: 94 - protein, 9 aa, Artificial
  peptide
RLSNDTVGL

SEQ ID NO: 95 - protein, 9 aa, Artificial
  peptide
RMSNDTVEI

SEQ ID NO: 96 - protein, 9 aa, Artificial
  peptide
TLSNDTVWL

SEQ ID NO: 97 - protein, 9 aa, Artificial
  peptide
ALLGPWLIV

SEQ ID NO: 98 - protein, 9 aa, Artificial
  peptide
FLLGPWLCL

SEQ ID NO: 99 - protein, 9 aa, Artificial
  peptide
KLLGPWLSV

SEQ ID NO: 100 - protein, 9 aa, Artificial
  peptide
LLLGPWLLL

SEQ ID NO: 101 - protein, 9 aa, Artificial
  peptide
YLLGPWLLV

SEQ ID NO: 102 - protein, 9 aa, Artificial
  peptide
ILILAICGV

SEQ ID NO: 103 - protein, 9 aa, Artificial
  peptide
IMILAICLV

SEQ ID NO: 104 - protein, 9 aa, Artificial
  peptide
RLILAICGL

SEQ ID NO: 105 - protein, 9 aa, Artificial
  peptide
YLILAICGV

SEQ ID NO: 106 - protein, 9 aa, Artificial
  peptide
KIFEHPELL

SEQ ID NO: 107 - protein, 9 aa, Artificial
  peptide
LIFEHPERV

SEQ ID NO: 108 - protein, 9 aa, Artificial
  peptide
RVFEHPELV

SEQ ID NO: 109 - protein, 9 aa, Artificial
  peptide
YVFEHPELL

SEQ ID NO: 110 - protein, 9 aa, Artificial
  peptide
YIFEHPETA

SEQ ID NO: 111 - protein, 9 aa, Artificial
  peptide
ALAFVPLAV

SEQ ID NO: 112 - protein, 9 aa, Artificial
  peptide
ALAFVPLSV

SEQ ID NO: 113 - protein, 9 aa, Artificial
  peptide
FLAFVPLIL

SEQ ID NO: 114 - protein, 9 aa, Artificial
  peptide
FLAFVPLQL

SEQ ID NO: 115 - protein, 9 aa, Artificial
  peptide
FLAFVPLVL

SEQ ID NO: 116 - protein, 9 aa, Artificial
  peptide
FMAFVPLQL

SEQ ID NO: 117 - protein, 9 aa, Artificial
  peptide
GMAFVPLLL

SEQ ID NO: 118 - protein, 9 aa, Artificial
  peptide
HLAFVPLLV

SEQ ID NO: 119 - protein, 9 aa, Artificial
  peptide
ILAFVPLYL

SEQ ID NO: 120 - protein, 9 aa, Artificial
  peptide
IMAFVPLAV

SEQ ID NO: 121 - protein, 9 aa, Artificial
  peptide
IMAFVPLIV

SEQ ID NO: 122 - protein, 9 aa, Artificial
  peptide
IMAFVPLVV

SEQ ID NO: 123 - protein, 9 aa, Artificial
  peptide
LLAFVPLAL

SEQ ID NO: 124 - protein, 9 aa, Artificial
  peptide
LLAFVPLDV

SEQ ID NO: 125 - protein, 9 aa, Artificial
  peptide
LLAFVPLML

SEQ ID NO: 126 - protein, 9 aa, Artificial
  peptide
LLAFVPLSL

SEQ ID NO: 127 - protein, 9 aa, Artificial
  peptide
LMAFVPLTL

SEQ ID NO: 128 - protein, 9 aa, Artificial
  peptide
TLAFVPLAV

SEQ ID NO: 129 - protein, 9 aa, Artificial
  peptide
VLAFVPLLV

SEQ ID NO: 130 - protein, 9 aa, Artificial
  peptide
VMAFVPLVV

SEQ ID NO: 131 - protein, 9 aa, Artificial
  peptide
FLYFGMLLL

SEQ ID NO: 132 - protein, 9 aa, Artificial
  peptide
GLYFGMLHM

SEQ ID NO: 133 - protein, 9 aa, Artificial
  peptide
LLYFGMLGL

SEQ ID NO: 134 - protein, 9 aa, Artificial
  peptide
LLYFGMLLL

SEQ ID NO: 135 - protein, 9 aa, Artificial
  peptide
TMYFGMLYL

SEQ ID NO: 136 - protein, 9 aa, Artificial
  peptide
VLYFGMLLI

SEQ ID NO: 137 - protein, 9 aa, Artificial
  peptide
CLIDKTSVV

SEQ ID NO: 138 - protein, 9 aa, Artificial
  peptide
FLIDKTSAA

SEQ ID NO: 139 - protein, 9 aa, Artificial
  peptide
ILIDKTSGA

SEQ ID NO: 140 - protein, 9 aa, Artificial
  peptide
ILIDKTSGV

SEQ ID NO: 141 - protein, 9 aa, Artificial
  peptide
IMIDKTSTV

SEQ ID NO: 142 - protein, 9 aa, Artificial
  peptide
VIIDKTSSV

SEQ ID NO: 143 - protein, 9 aa, Artificial
  peptide
VLIDKTSQL

SEQ ID NO: 144 - protein, 9 aa, Artificial
  peptide
VLIDKTSSV

SEQ ID NO: 145 - protein, 9 aa, Artificial
  peptide
YLIDKTSNI

SEQ ID NO: 146 - protein, 9 aa, Artificial
  peptide
YLIDKTSNL

SEQ ID NO: 147 - protein, 9 aa, Artificial
  peptide
YLIDKTSTV

SEQ ID NO: 148 - protein, 9 aa, Artificial
  peptide
FILLFATHV

SEQ ID NO: 149 - protein, 9 aa, Artificial
  peptide
FLLLFATSV

SEQ ID NO: 150 - protein, 9 aa, Artificial
  peptide
LLLLFATAV

SEQ ID NO: 151 - protein, 9 aa, Artificial
  peptide
LLLLFATSV

SEQ ID NO: 152 - protein, 9 aa, Artificial
  peptide
LMLLFATSV

SEQ ID NO: 153 - protein, 9 aa, Artificial
  peptide
MMLLFATLL

SEQ ID NO: 154 - protein, 9 aa, Artificial
  peptide
YLLLFATNV

SEQ ID NO: 155 - protein, 9 aa, Artificial
  peptide
YLLLFATYL

SEQ ID NO: 156 - protein, 9 aa, Artificial
  peptide
ILVGICLGV

SEQ ID NO: 157 - protein, 9 aa, Artificial
  peptide
SIVGICLNV

SEQ ID NO: 158 - protein, 9 aa, Artificial
  peptide
KLIKYFLKV

SEQ ID NO: 159 - protein, 9 aa, Artificial
  peptide
KLIKYFLVV

SEQ ID NO: 160 - protein, 9 aa, Artificial
  peptide
MMIKYFLCV

SEQ ID NO: 161 - protein, 9 aa, Artificial
  peptide
NLIKYFLYV

SEQ ID NO: 162 - protein, 9 aa, Artificial
  peptide
SLIKYFLSI

SEQ ID NO: 163 - protein, 9 aa, Artificial
  peptide
ALVLALVGV

SEQ ID NO: 164 - protein, 9 aa, Artificial
  peptide
ALVLALVPV

SEQ ID NO: 165 - protein, 9 aa, Artificial
  peptide
GLVLALVGV

SEQ ID NO: 166 - protein, 9 aa, Artificial
  peptide
NLVLALVEV

SEQ ID NO: 167 - protein, 9 aa, Artificial
  peptide
SLVLALVGV

SEQ ID NO: 168 - protein, 9 aa, Artificial
  peptide
SLVLALVSV

SEQ ID NO: 169 - protein, 9 aa, Artificial
  peptide
SLVLALVYV

SEQ ID NO: 170 - protein, 9 aa, Artificial
  peptide
TLVLALVSV

SEQ ID NO: 171 - protein, 9 aa, Artificial
  peptide
ALALVLALL

SEQ ID NO: 172 - protein, 9 aa, Artificial
  peptide
ALALVLAML

SEQ ID NO: 173 - protein, 9 aa, Artificial
  peptide
ALALVLATV

SEQ ID NO: 174 - protein, 9 aa, Artificial
  peptide
FLALVLAAA

SEQ ID NO: 175 - protein, 9 aa, Artificial
  peptide
FLALVLAAL

SEQ ID NO: 176 - protein, 9 aa, Artificial
  peptide
FLALVLAGL

SEQ ID NO: 177 - protein, 9 aa, Artificial
  peptide
FLALVLAGV

SEQ ID NO: 178 - protein, 9 aa, Artificial
  peptide
FLALVLALL

SEQ ID NO: 179 - protein, 9 aa, Artificial
  peptide
FLALVLAML

SEQ ID NO: 180 - protein, 9 aa, Artificial
  peptide
FLALVLATL

SEQ ID NO: 181 - protein, 9 aa, Artificial
  peptide
GLALVLAAI

SEQ ID NO: 182 - protein, 9 aa, Artificial
  peptide
GLALVLAAL

SEQ ID NO: 183 - protein, 9 aa, Artificial
  peptide
GLALVLAAV

SEQ ID NO: 184 - protein, 9 aa, Artificial
  peptide
GLALVLALL

SEQ ID NO: 185 - protein, 9 aa, Artificial
  peptide
GLALVLALV

SEQ ID NO: 186 - protein, 9 aa, Artificial
  peptide
GLALVLANI

SEQ ID NO: 187 - protein, 9 aa, Artificial
  peptide
GLALVLATL

SEQ ID NO: 188 - protein, 9 aa, Artificial
  peptide
GLALVLATV

SEQ ID NO: 189 - protein, 9 aa, Artificial
  peptide
GLALVLAVV

SEQ ID NO: 190 - protein, 9 aa, Artificial
  peptide
GMALVLAAV

SEQ ID NO: 191 - protein, 9 aa, Artificial
  peptide
ILALVLAMV

SEQ ID NO: 192 - protein, 9 aa, Artificial
  peptide
ILALVLARV

SEQ ID NO: 193 - protein, 9 aa, Artificial
  peptide
ILALVLAYL

SEQ ID NO: 194 - protein, 9 aa, Artificial
  peptide
KLALVLAML

SEQ ID NO: 195 - protein, 9 aa, Artificial
  peptide
LLALVLAEV

SEQ ID NO: 196 - protein, 9 aa, Artificial
  peptide
MLALVLAGL

SEQ ID NO: 197 - protein, 9 aa, Artificial
  peptide
SLALVLALL

SEQ ID NO: 198 - protein, 9 aa, Artificial
  peptide
SLALVLALV

SEQ ID NO: 199 - protein, 9 aa, Artificial
  peptide
SLALVLAML

SEQ ID NO: 200 - protein, 9 aa, Artificial
  peptide
VLALVLAEL

SEQ ID NO: 201 - protein, 9 aa, Artificial
  peptide
VLALVLAEV

SEQ ID NO: 202 - protein, 9 aa, Artificial
  peptide
VLALVLAGV

SEQ ID NO: 203 - protein, 9 aa, Artificial
  peptide
VLALVLALV

SEQ ID NO: 204 - protein, 9 aa, Artificial
  peptide
VLALVLAMV

SEQ ID NO: 205 - protein, 9 aa, Artificial
  peptide
VLALVLATV

SEQ ID NO: 206 - protein, 9 aa, Artificial
  peptide
YLALVLAFL

SEQ ID NO: 207 - protein, 9 aa, Artificial
  peptide
YLALVLALI

SEQ ID NO: 208 - protein, 9 aa, Artificial
  peptide
YLALVLALL

SEQ ID NO: 209 - protein, 9 aa, Artificial
  peptide
YLALVLAML

SEQ ID NO: 210 - protein, 9 aa, Artificial
  peptide
ALFGAPAAV

SEQ ID NO: 211 - protein, 9 aa, Artificial
  peptide
ALFGAPAKL

SEQ ID NO: 212 - protein, 9 aa, Artificial
  peptide
FLFGAPASA

SEQ ID NO: 213 - protein, 9 aa, Artificial
  peptide
GLFGAPAFI

SEQ ID NO: 214 - protein, 9 aa, Artificial
  peptide
LLFGAPAAL

SEQ ID NO: 215 - protein, 9 aa, Artificial
  peptide
LLFGAPAGI

SEQ ID NO: 216 - protein, 9 aa, Artificial
  peptide
LLFGAPAGL

SEQ ID NO: 217 - protein, 9 aa, Artificial
  peptide
LLFGAPAGV

SEQ ID NO: 218 - protein, 9 aa, Artificial
  peptide
LLFGAPALL

SEQ ID NO: 219 - protein, 9 aa, Artificial
  peptide
LMFGAPAFV

SEQ ID NO: 220 - protein, 9 aa, Artificial
  peptide
LMFGAPALV

SEQ ID NO: 221 - protein, 9 aa, Artificial
  peptide
MLFGAPAEA

SEQ ID NO: 222 - protein, 9 aa, Artificial
  peptide
SMFGAPAHV

SEQ ID NO: 223 - protein, 9 aa, Artificial
  peptide
VLFGAPANL

SEQ ID NO: 224 - protein, 9 aa, Artificial
  peptide
VLFGAPAYL

SEQ ID NO: 225 - protein, 9 aa, Artificial
  peptide
YLFGAPAAA

SEQ ID NO: 226 - protein, 9 aa, Artificial
  peptide
FLPGLLFSV

SEQ ID NO: 227 - protein, 9 aa, Artificial
  peptide
FMPGLLFGA

SEQ ID NO: 228 - protein, 9 aa, Artificial
  peptide
FVPGLLFGV

SEQ ID NO: 229 - protein, 9 aa, Artificial
  peptide
GLPGLLFEL

SEQ ID NO: 230 - protein, 9 aa, Artificial
  peptide
ILPGLLFAI

SEQ ID NO: 231 - protein, 9 aa, Artificial
  peptide
ILPGLLFGL

SEQ ID NO: 232 - protein, 9 aa, Artificial
  peptide
ILPGLLFLI

SEQ ID NO: 233 - protein, 9 aa, Artificial
  peptide
ILPGLLFSL

SEQ ID NO: 234 - protein, 9 aa, Artificial
  peptide
ILPGLLFYI

SEQ ID NO: 235 - protein, 9 aa, Artificial
  peptide
ILPGLLFYM

SEQ ID NO: 236 - protein, 9 aa, Artificial
  peptide
IMPGLLFHI

SEQ ID NO: 237 - protein, 9 aa, Artificial
  peptide
IMPGLLFQV

SEQ ID NO: 238 - protein, 9 aa, Artificial
  peptide
IMPGLLFYV

SEQ ID NO: 239 - protein, 9 aa, Artificial
  peptide
KLPGLLFHA

SEQ ID NO: 240 - protein, 9 aa, Artificial
  peptide
KLPGLLFSV

SEQ ID NO: 241 - protein, 9 aa, Artificial
  peptide
LLPGLLFGL

SEQ ID NO: 242 - protein, 9 aa, Artificial
  peptide
LLPGLLFTL

SEQ ID NO: 243 - protein, 9 aa, Artificial
  peptide
LLPGLLFVV

SEQ ID NO: 244 - protein, 9 aa, Artificial
  peptide
MLPGLLFAL

SEQ ID NO: 245 - protein, 9 aa, Artificial
  peptide
MLPGLLFGL

SEQ ID NO: 246 - protein, 9 aa, Artificial
  peptide
MLPGLLFKV

SEQ ID NO: 247 - protein, 9 aa, Artificial
  peptide
MLPGLLFVV

SEQ ID NO: 248 - protein, 9 aa, Artificial
  peptide
PLPGLLFSV

SEQ ID NO: 249 - protein, 9 aa, Artificial
  peptide
RMPGLLFKV

SEQ ID NO: 250 - protein, 9 aa, Artificial
  peptide
SLPGLLFFL

SEQ ID NO: 251 - protein, 9 aa, Artificial
  peptide
SLPGLLFTL

SEQ ID NO: 252 - protein, 9 aa, Artificial
  peptide
SLPGLLFVV

SEQ ID NO: 253 - protein, 9 aa, Artificial
  peptide
TLPGLLFPA

SEQ ID NO: 254 - protein, 9 aa, Artificial
  peptide
TLPGLLFPV

SEQ ID NO: 255 - protein, 9 aa, Artificial
  peptide
VLPGLLFGV

SEQ ID NO: 256 - protein, 9 aa, Artificial
  peptide
VLPGLLFYV

SEQ ID NO: 257 - protein, 9 aa, Artificial
  peptide
YLPGLLFLM

SEQ ID NO: 258 - protein, 9 aa, Homo sapiens
FLLFLTPME

SEQ ID NO: 259 - protein, 9 aa, Homo sapiens
KLSLGLPGL

SEQ ID NO: 260 - protein, 9 aa, Homo sapiens
SLVGILHLQ

SEQ ID NO: 261 - protein, 9 aa, Homo sapiens
TLAYLIFCL

SEQ ID NO: 262 - protein, 9 aa, Homo sapiens
QQMGGFYLC

SEQ ID NO: 263 - protein, 9 aa, Homo sapiens
IALGGLLMI

SEQ ID NO: 264 - protein, 9 aa, Homo sapiens
IMNSLSLFA

SEQ ID NO: 265 - protein, 9 aa, Homo sapiens
LMIPAGIYA

SEQ ID NO: 266 - protein, 9 aa, Homo sapiens
SLFLGILSV

SEQ ID NO: 267 - protein, 9 aa, Homo sapiens
FLSNDTVQL

SEQ ID NO: 268 - protein, 9 aa, Homo sapiens
HLLGPWLLL

SEQ ID NO: 269 - protein, 9 aa, Homo sapiens
ILILAICGL

SEQ ID NO: 270 - protein, 9 aa, Homo sapiens
WVFEHPETL

SEQ ID NO: 271 - protein, 9 aa, Homo sapiens
GLAFVPLQI

SEQ ID NO: 272 - protein, 9 aa, Homo sapiens
GLYFGMLLL

SEQ ID NO: 273 - protein, 9 aa, Homo sapiens
ILIDKTSFV

SEQ ID NO: 274 - protein, 9 aa, Homo sapiens
LLLLFATQI

SEQ ID NO: 275 - protein, 9 aa, Homo sapiens
SIVGICLGV

SEQ ID NO: 276 - protein, 9 aa, Homo sapiens
SIVGICLGV

SEQ ID NO: 277 - protein, 9 aa, Homo sapiens
ALVLALVLV

SEQ ID NO: 278 - protein, 9 aa, Homo sapiens
GLALVLALV

SEQ ID NO: 279 - protein, 9 aa, Homo sapiens
LLFGAPALL

SEQ ID NO: 280 - protein, 9 aa, Homo sapiens
PLPGLLFGA

SEQ ID NO: 281 - protein, 5 aa, Homo sapiens
LFLTP

SEQ ID NO: 282 - protein, 5 aa, Homo sapiens
SLGLP

SEQ ID NO: 283 - protein, 5 aa, Homo sapiens
VGILH

SEQ ID NO: 284 - protein, 5 aa, Homo sapiens
AYLIF

SEQ ID NO: 285 - protein, 5 aa, Homo sapiens
MGGFY

SEQ ID NO: 286 - protein, 5 aa, Homo sapiens
LGGLL

SEQ ID NO: 287 - protein, 5 aa, Homo sapiens
NSLSL

SEQ ID NO: 288 - protein, 5 aa, Homo sapiens
IPAGI

SEQ ID NO: 289 - protein, 5 aa, Homo sapiens
FLGIL

SEQ ID NO: 290 - protein, 5 aa, Homo sapiens
SNDTV

SEQ ID NO: 291 - protein, 5 aa, Homo sapiens
LGPWL

SEQ ID NO: 292 - protein, 5 aa, Homo sapiens
ILAIC

SEQ ID NO: 293 - protein, 5 aa, Homo sapiens
FEHPE

SEQ ID NO: 294 - protein, 5 aa, Homo sapiens
AFVPL

SEQ ID NO: 295 - protein, 5 aa, Homo sapiens
YFGML

SEQ ID NO: 296 - protein, 5 aa, Homo sapiens
IDKTS

SEQ ID NO: 297 - protein, 5 aa, Homo sapiens
LLFAT

SEQ ID NO: 298 - protein, 5 aa, Homo sapiens
VGICL

SEQ ID NO: 299 - protein, 5 aa, Homo sapiens
IKYFL

SEQ ID NO: 300 - protein, 5 aa, Homo sapiens
VLALV

SEQ ID NO: 301 - protein, 5 aa, Homo sapiens
ALVLA

SEQ ID NO: 302 - protein, 5 aa, Homo sapiens
FGAPA

SEQ ID NO: 303 - protein, 5 aa, Homo sapiens
PGLLF

SEQ ID NO: 304 - protein, 9 aa, Artificial
  peptide
  misc_feature (1)..(2): Xaa can be any naturally occurring amino acid
  misc_feature (8)..(9): Xaa can be any naturally occurring amino acid
XXLFLTPXX

SEQ ID NO: 305 - protein, 9 aa, Artificial
  peptide
  misc_feature (1)..(2): Xaa can be any naturally occurring amino acid
  misc_feature (8)..(9): Xaa can be any naturally occurring amino acid
XXSLGLPXX

SEQ ID NO: 306 - protein, 9 aa, Artificial
  peptide
  misc_feature (1)..(2): Xaa can be any naturally occurring amino acid
  misc_feature (8)..(9): Xaa can be any naturally occurring amino acid
XXVGILHXX

SEQ ID NO: 307 - protein, 9 aa, Artificial
  peptide
  misc_feature (1)..(2): Xaa can be any naturally occurring amino acid
  misc_feature (8)..(9): Xaa can be any naturally occurring amino acid
XXAYLIFXX

SEQ ID NO: 308 - protein, 9 aa, Artificial
  peptide
  misc_feature (1)..(2): Xaa can be any naturally occurring amino acid
  misc_feature (8)..(9): Xaa can be any naturally occurring amino acid
XXMGGFYXX

SEQ ID NO: 309 - protein, 9 aa, Artificial
  peptide
  misc_feature (1)..(2): Xaa can be any naturally occurring amino acid
  misc_feature (8)..(9): Xaa can be any naturally occurring amino acid
XXLGGLLXX

SEQ ID NO: 310 - protein, 9 aa, Artificial
  peptide
  misc_feature (1)..(2): Xaa can be any naturally occurring amino acid
  misc_feature (8)..(9): Xaa can be any naturally occurring amino acid
XXNSLSLXX

SEQ ID NO: 311 - protein, 9 aa, Artificial
  peptide
  misc_feature (1)..(2): Xaa can be any naturally occurring amino acid
  misc_feature (8)..(9): Xaa can be any naturally occurring amino acid
XXIPAGIXX

SEQ ID NO: 312 - protein, 9 aa, Artificial
  peptide
  misc_feature (1)..(2): Xaa can be any naturally occurring amino acid
  misc_feature (8)..(9): Xaa can be any naturally occurring amino acid
XXFLGILXX

SEQ ID NO: 313 - protein, 9 aa, Artificial
  peptide
  misc_feature (1)..(2): Xaa can be any naturally occurring amino acid
  misc_feature (8)..(9): Xaa can be any naturally occurring amino acid
XXSNDTVXX

SEQ ID NO: 314 - protein, 9 aa, Artificial
  XXLGPWLXX
  misc_feature (1)..(2): Xaa can be any naturally occurring amino acid
  misc_feature (8)..(9): Xaa can be any naturally occurring amino acid
XXLGPWLXX

SEQ ID NO: 315 - protein, 9 aa, Artificial
  peptide
  misc_feature (1)..(2): Xaa can be any naturally occurring amino acid
  misc_feature (8)..(9): Xaa can be any naturally occurring amino acid
XXILAICXX

SEQ ID NO: 316 - protein, 9 aa, Artificial
  peptide
  misc_feature (1)..(2): Xaa can be any naturally occurring amino acid
  misc_feature (8)..(9): Xaa can be any naturally occurring amino acid
XXFEHPEXX

SEQ ID NO: 317 - protein, 9 aa, Artificial
  peptide
  misc_feature (1)..(2): Xaa can be any naturally occurring amino acid
  misc_feature (8)..(9): Xaa can be any naturally occurring amino acid
XXAFVPLXX

SEQ ID NO: 318 - protein, 9 aa, Artificial
  peptide
  misc_feature (1)..(2): Xaa can be any naturally occurring amino acid
  misc_feature (8)..(9): Xaa can be any naturally occurring amino acid
XXYFGMLXX

SEQ ID NO: 319 - protein, 9 aa, Artificial
  peptide
  misc_feature (1)..(2): Xaa can be any naturally occurring amino acid
  misc_feature (8)..(9): Xaa can be any naturally occurring amino acid
XXIDKTSXX

SEQ ID NO: 320 - protein, 9 aa, Artificial
  peptide
  misc_feature (1)..(2): Xaa can be any naturally occurring amino acid
  misc_feature (8)..(9): Xaa can be any naturally occurring amino acid
XXLLFATXX

SEQ ID NO: 321 - protein, 9 aa, Artificial
  peptide
  misc_feature (1)..(2): Xaa can be any naturally occurring amino acid
  misc_feature (8)..(9): Xaa can be any naturally occurring amino acid
XXVGICLXX

SEQ ID NO: 322 - protein, 9 aa, Artificial
  peptide
  misc_feature (1)..(2): Xaa can be any naturally occurring amino acid
  misc_feature (8)..(9): Xaa can be any naturally occurring amino acid
XXIKYFLXX

SEQ ID NO: 323 - protein, 9 aa, Artificial
  peptide
  misc_feature (1)..(2): Xaa can be any naturally occurring amino acid
  misc_feature (8)..(9): Xaa can be any naturally occurring amino acid
XXVLALVXX

SEQ ID NO: 324 - protein, 9 aa, Artificial
  peptide
  misc_feature (1)..(2): Xaa can be any naturally occurring amino acid
  misc_feature (8)..(9): Xaa can be any naturally occurring amino acid
XXALVLAXX

SEQ ID NO: 325 - protein, 9 aa, Artificial
  peptide
  misc_feature (1)..(2): Xaa can be any naturally occurring amino acid
  misc_feature (8)..(9): Xaa can be any naturally occurring amino acid
XXFGAPAXX

SEQ ID NO: 326 - protein, 9 aa, Artificial
  peptide
  misc_feature (1)..(2): Xaa can be any naturally occurring amino acid
  misc_feature (8)..(9): Xaa can be any naturally occurring amino acid
XXPGLLFXX

SEQ ID NO: 327 - protein, 9 aa, Artificial
  peptide
  misc_feature (8)..(8): Xaa can be any naturally occurring amino acid
FLLFLTPXL

SEQ ID NO: 328 - protein, 9 aa, Artificial
  peptide
  misc_feature (2)..(2): Xaa can be any naturally occurring amino acid
  misc_feature (8)..(9): Xaa can be any naturally occurring amino acid
FXLFLTPXX

SEQ ID NO: 329 - protein, 9 aa, Artificial
  peptide
  misc_feature (8)..(9): Xaa can be any naturally occurring amino acid
GLLFLTPXX

SEQ ID NO: 330 - protein, 9 aa, Artificial
  peptide
  misc_feature (8)..(9): Xaa can be any naturally occurring amino acid
TLLFLTPXX

SEQ ID NO: 331 - protein, 9 aa, Artificial
  peptide
  misc_feature (1)..(1): Xaa can be any naturally occurring amino acid
XLLFLTPLL

SEQ ID NO: 332 - protein, 9 aa, Artificial
  peptide
  misc_feature (1)..(1): Xaa can be any naturally occurring amino acid
XLLFLTPML

SEQ ID NO: 333 - protein, 9 aa, Artificial
  peptide
  misc_feature (1)..(1): Xaa can be any naturally occurring amino acid
  misc_feature (8)..(8): Xaa can be any naturally occurring amino acid
XLLFLTPXL

SEQ ID NO: 334 - protein, 9 aa, Artificial
  peptide
  misc_feature (8)..(8): Xaa can be any naturally occurring amino acid
ALSLGLPXL

SEQ ID NO: 335 - protein, 9 aa, Artificial
  peptide
  misc_feature (8)..(8): Xaa can be any naturally occurring amino acid
AMSLGLPXL

SEQ ID NO: 336 - protein, 9 aa, Artificial
  peptide
  misc_feature (8)..(8): Xaa can be any naturally occurring amino acid
FLSLGLPXL

SEQ ID NO: 337 - protein, 9 aa, Artificial
  peptide
  misc_feature (8)..(8): Xaa can be any naturally occurring amino acid
LLSLGLPXL

SEQ ID NO: 338 - protein, 9 aa, Artificial
  peptide
  misc_feature (8)..(8): Xaa can be any naturally occurring amino acid
SLSLGLPXL

SEQ ID NO: 339 - protein, 9 aa, Artificial
  peptide
  misc_feature (8)..(9): Xaa can be any naturally occurring amino acid
VLSLGLPXX

SEQ ID NO: 340 - protein, 9 aa, Artificial
  peptide
  misc_feature (1)..(1): Xaa can be any naturally occurring amino acid
XLSLGLPGL

SEQ ID NO: 341 - protein, 9 aa, Artificial
  peptide
  misc_feature (1)..(1): Xaa can be any naturally occurring amino acid
XLSLGLPIL

SEQ ID NO: 342 - protein, 9 aa, Artificial
  peptide
  misc_feature (1)..(1): Xaa can be any naturally occurring amino acid
XLSLGLPKL

SEQ ID NO: 343 - protein, 9 aa, Artificial
  peptide
  misc_feature (1)..(1): Xaa can be any naturally occurring amino acid
  misc_feature (8)..(8): Xaa can be any naturally occurring amino acid
XLSLGLPXL

SEQ ID NO: 344 - protein, 9 aa, Artificial
  peptide
  misc_feature (1)..(1): Xaa can be any naturally occurring amino acid
  misc_feature (8)..(9): Xaa can be any naturally occurring amino acid
XLVGILHXX

SEQ ID NO: 345 - protein, 9 aa, Artificial
  peptide
  misc_feature (8)..(8): Xaa can be any naturally occurring amino acid
FLAYLIFXL

SEQ ID NO: 346 - protein, 9 aa, Artificial
  peptide
  misc_feature (1)..(1): Xaa can be any naturally occurring amino acid
  misc_feature (8)..(8): Xaa can be any naturally occurring amino acid
XLAYLIFXL

SEQ ID NO: 347 - protein, 9 aa, Artificial
  peptide
  misc_feature (8)..(9): Xaa can be any naturally occurring amino acid
ALLGGLLXX

SEQ ID NO: 348 - protein, 9 aa, Artificial
  peptide
  misc_feature (2)..(2): Xaa can be any naturally occurring amino acid
AXLGGLLLI

SEQ ID NO: 349 - protein, 9 aa, Artificial
  peptide
  misc_feature (2)..(2): Xaa can be any naturally occurring amino acid
  misc_feature (8)..(8): Xaa can be any naturally occurring amino acid
FXLGGLLXV

SEQ ID NO: 350 - protein, 9 aa, Artificial
  peptide
  misc_feature (8)..(9): Xaa can be any naturally occurring amino acid
GMLGGLLXX

SEQ ID NO: 351 - protein, 9 aa, Artificial
  peptide
  misc_feature (1)..(1): Xaa can be any naturally occurring amino acid
  misc_feature (8)..(8): Xaa can be any naturally occurring amino acid
XLLGGLLXI

SEQ ID NO: 352 - protein, 9 aa, Artificial
  peptide
  misc_feature (8)..(9): Xaa can be any naturally occurring amino acid
SLLGGLLXX

SEQ ID NO: 353 - protein, 9 aa, Artificial
  peptide
  misc_feature (2)..(2): Xaa can be any naturally occurring amino acid
SXLGGLLLI

SEQ ID NO: 354 - protein, 9 aa, Artificial
  peptide
  misc_feature (2)..(2): Xaa can be any naturally occurring amino acid
YXLGGLLMV

SEQ ID NO: 355 - protein, 9 aa, Artificial
  peptide
  misc_feature (2)..(2): Xaa can be any naturally occurring amino acid
  misc_feature (8)..(8): Xaa can be any naturally occurring amino acid
YXLGGLLXV

SEQ ID NO: 356 - protein, 9 aa, Artificial
  peptide
  misc_feature (1)..(1): Xaa can be any naturally occurring amino acid
XLLGGLLLI

SEQ ID NO: 357 - protein, 9 aa, Artificial
  peptide
  misc_feature (1)..(1): Xaa can be any naturally occurring amino acid
XMLGGLLLI

SEQ ID NO: 358 - protein, 9 aa, Artificial
  peptide
  misc_feature (1)..(2): Xaa can be any naturally occurring amino acid
XXLGGLLMI

SEQ ID NO: 359 - protein, 9 aa, Artificial
  peptide
  misc_feature (1)..(2): Xaa can be any naturally occurring amino acid
XXLGGLLML

SEQ ID NO: 360 - protein, 9 aa, Artificial
  peptide
  misc_feature (1)..(2): Xaa can be any naturally occurring amino acid
XXLGGLLMV

SEQ ID NO: 361 - protein, 9 aa, Artificial
  peptide
  misc_feature (8)..(9): Xaa can be any naturally occurring amino acid
ILNSLSLXX

SEQ ID NO: 362 - protein, 9 aa, Artificial
  peptide
  misc_feature (1)..(1): Xaa can be any naturally occurring amino acid
  misc_feature (8)..(8): Xaa can be any naturally occurring amino acid
XLNSLSLXL

SEQ ID NO: 363 - protein, 9 aa, Artificial
  peptide
  misc_feature (1)..(1): Xaa can be any naturally occurring amino acid
  misc_feature (8)..(9): Xaa can be any naturally occurring amino acid
XMNSLSLXX

SEQ ID NO: 364 - protein, 9 aa, Artificial
  peptide
  misc_feature (1)..(2): Xaa can be any naturally occurring amino acid
  misc_feature (8)..(8): Xaa can be any naturally occurring amino acid
XXNSLSLXI

SEQ ID NO: 365 - protein, 9 aa, Artificial
  peptide
  misc_feature (8)..(9): Xaa can be any naturally occurring amino acid
LLIPAGIXX

SEQ ID NO: 366 - protein, 9 aa, Artificial
  peptide
  misc_feature (2)..(2): Xaa can be any naturally occurring amino acid
  misc_feature (8)..(9): Xaa can be any naturally occurring amino acid
MXIPAGIXX

SEQ ID NO: 367 - protein, 9 aa, Artificial
  peptide
  misc_feature (1)..(1): Xaa can be any naturally occurring amino acid
  misc_feature (8)..(8): Xaa can be any naturally occurring amino acid
XLIPAGIXL

SEQ ID NO: 368 - protein, 9 aa, Artificial
  peptide
  misc_feature (1)..(1): Xaa can be any naturally occurring amino acid
  misc_feature (8)..(9): Xaa can be any naturally occurring amino acid
XMIPAGIXX

SEQ ID NO: 369 - protein, 9 aa, Artificial
  peptide
  misc_feature (1)..(2): Xaa can be any naturally occurring amino acid
XXIPAGIAV

SEQ ID NO: 370 - protein, 9 aa, Artificial
  peptide
  misc_feature (8)..(8): Xaa can be any naturally occurring amino acid
FLFLGILXL

SEQ ID NO: 371 - protein, 9 aa, Artificial
  peptide
  misc_feature (8)..(8): Xaa can be any naturally occurring amino acid
YLFLGILXL

SEQ ID NO: 372 - protein, 9 aa, Artificial
  peptide
  misc_feature (8)..(9): Xaa can be any naturally occurring amino acid
YLFLGILXX

SEQ ID NO: 373 - protein, 9 aa, Artificial
  peptide
  misc_feature (1)..(1): Xaa can be any naturally occurring amino acid
XLFLGILGL

SEQ ID NO: 374 - protein, 9 aa, Artificial
  peptide
  misc_feature (1)..(1): Xaa can be any naturally occurring amino acid
  misc_feature (9)..(9): Xaa can be any naturally occurring amino acid
XLFLGILSX

SEQ ID NO: 375 - protein, 9 aa, Artificial
  peptide
  misc_feature (8)..(8): Xaa can be any naturally occurring amino acid
FLSNDTVXL

SEQ ID NO: 376 - protein, 9 aa, Artificial
  peptide
  misc_feature (8)..(9): Xaa can be any naturally occurring amino acid
FLSNDTVXX

SEQ ID NO: 377 - protein, 9 aa, Artificial
  peptide
  misc_feature (2)..(2): Xaa can be any naturally occurring amino acid
  misc_feature (8)..(9): Xaa can be any naturally occurring amino acid
FXSNDTVXX

SEQ ID NO: 378 - protein, 9 aa, Artificial
  peptide
  misc_feature (1)..(1): Xaa can be any naturally occurring amino acid
  misc_feature (8)..(9): Xaa can be any naturally occurring amino acid
XMSNDTVXX

SEQ ID NO: 379 - protein, 9 aa, Artificial
  peptide
  misc_feature (1)..(1): Xaa can be any naturally occurring amino acid
XLSNDTVWL

SEQ ID NO: 380 - protein, 9 aa, Artificial
  peptide
  misc_feature (1)..(1): Xaa can be any naturally occurring amino acid
  misc_feature (8)..(8): Xaa can be any naturally occurring amino acid
XLSNDTVXL

SEQ ID NO: 381 - protein, 9 aa, Artificial
  peptide
  misc_feature (1)..(1): Xaa can be any naturally occurring amino acid
  misc_feature (8)..(8): Xaa can be any naturally occurring amino acid
XLLGPWLXL

SEQ ID NO: 382 - protein, 9 aa, Artificial
  peptide
  misc_feature (1)..(1): Xaa can be any naturally occurring amino acid
  misc_feature (8)..(8): Xaa can be any naturally occurring amino acid
XLLGPWLXV

SEQ ID NO: 383 - protein, 9 aa, Artificial
  peptide
  misc_feature (1)..(1): Xaa can be any naturally occurring amino acid
  misc_feature (8)..(9): Xaa can be any naturally occurring amino acid
XLLGPWLXX

SEQ ID NO: 384 - protein, 9 aa, Artificial
  peptide
  misc_feature (2)..(2): Xaa can be any naturally occurring amino acid
  misc_feature (8)..(8): Xaa can be any naturally occurring amino acid
IXILAICXV

SEQ ID NO: 385 - protein, 9 aa, Artificial
  peptide
  misc_feature (1)..(1): Xaa can be any naturally occurring amino acid
XLILAICGV

SEQ ID NO: 386 - protein, 9 aa, Artificial
  peptide
  misc_feature (1)..(1): Xaa can be any naturally occurring amino acid
  misc_feature (9)..(9): Xaa can be any naturally occurring amino acid
XLILAICGX

SEQ ID NO: 387 - protein, 9 aa, Artificial
  peptide
  misc_feature (1)..(1): Xaa can be any naturally occurring amino acid
  misc_feature (8)..(9): Xaa can be any naturally occurring amino acid
XIFEHPEXX

SEQ ID NO: 388 - protein, 9 aa, Artificial
  peptide
  misc_feature (1)..(2): Xaa can be any naturally occurring amino acid
XXFEHPELL

SEQ ID NO: 389 - protein, 9 aa, Artificial
  peptide
  misc_feature (1)..(2): Xaa can be any naturally occurring amino acid
  misc_feature (9)..(9): Xaa can be any naturally occurring amino acid
XXFEHPELX

SEQ ID NO: 390 - protein, 9 aa, Artificial
  peptide
  misc_feature (1)..(2): Xaa can be any naturally occurring amino acid
  misc_feature (8)..(9): Xaa can be any naturally occurring amino acid
XXFEHPEXX

SEQ ID NO: 391 - protein, 9 aa, Artificial
  peptide
  misc_feature (8)..(8): Xaa can be any naturally occurring amino acid
ALAFVPLXV

SEQ ID NO: 392 - protein, 9 aa, Artificial
  peptide
  misc_feature (8)..(8): Xaa can be any naturally occurring amino acid
FLAFVPLXL

SEQ ID NO: 393 - protein, 9 aa, Artificial
  peptide
  misc_feature (2)..(2): Xaa can be any naturally occurring amino acid
FXAFVPLQL

SEQ ID NO: 394 - protein, 9 aa, Artificial
  peptide
  misc_feature (8)..(8): Xaa can be any naturally occurring amino acid
IMAFVPLXV

SEQ ID NO: 395 - protein, 9 aa, Artificial
  peptide
  misc_feature (8)..(8): Xaa can be any naturally occurring amino acid
LLAFVPLXL

SEQ ID NO: 396 - protein, 9 aa, Artificial
  peptide
  misc_feature (8)..(9): Xaa can be any naturally occurring amino acid
LLAFVPLXX

SEQ ID NO: 397 - protein, 9 aa, Artificial
  peptide
  misc_feature (1)..(1): Xaa can be any naturally occurring amino acid
  misc_feature (8)..(8): Xaa can be any naturally occurring amino acid
XMAFVPLXV

SEQ ID NO: 398 - protein, 9 aa, Artificial
  peptide
  misc_feature (1)..(1): Xaa can be any naturally occurring amino acid
  misc_feature (8)..(8): Xaa can be any naturally occurring amino acid
XMAFVPLXL

SEQ ID NO: 399 - protein, 9 aa, Artificial
  peptide
  misc_feature (1)..(1): Xaa can be any naturally occurring amino acid
XLAFVPLAV

SEQ ID NO: 400 - protein, 9 aa, Artificial
  peptide
  misc_feature (1)..(1): Xaa can be any naturally occurring amino acid
  misc_feature (8)..(8): Xaa can be any naturally occurring amino acid
XLAFVPLXV

SEQ ID NO: 401 - protein, 9 aa, Artificial
  peptide
  misc_feature (1)..(2): Xaa can be any naturally occurring amino acid
XXAFVPLAV

SEQ ID NO: 402 - protein, 9 aa, Artificial
  peptide
  misc_feature (1)..(2): Xaa can be any naturally occurring amino acid
  misc_feature (8)..(8): Xaa can be any naturally occurring amino acid
XXAFVPLXL

SEQ ID NO: 403 - protein, 9 aa, Artificial
  peptide
  misc_feature (8)..(8): Xaa can be any naturally occurring amino acid
LLYFGMLXL

SEQ ID NO: 404 - protein, 9 aa, Artificial
  peptide
  misc_feature (1)..(1): Xaa can be any naturally occurring amino acid
  misc_feature (8)..(8): Xaa can be any naturally occurring amino acid
XLYFGMLXL

SEQ ID NO: 405 - protein, 9 aa, Artificial
  peptide
  misc_feature (1)..(1): Xaa can be any naturally occurring amino acid
  misc_feature (8)..(9): Xaa can be any naturally occurring amino acid
XLYFGMLXX

SEQ ID NO: 406 - protein, 10 aa, Artificial
  peptide
  misc_feature (1)..(2): Xaa can be any naturally occurring amino acid
  misc_feature (9)..(9): Xaa can be any naturally occurring amino acid
XXLYFGMLXL

SEQ ID NO: 407 - protein, 9 aa, Artificial
  peptide
  misc_feature (9)..(9): Xaa can be any naturally occurring amino acid
ILIDKTSGX

SEQ ID NO: 408 - protein, 9 aa, Artificial
  peptide
  misc_feature (2)..(2): Xaa can be any naturally occurring amino acid
  misc_feature (8)..(8): Xaa can be any naturally occurring amino acid
IXIDKTSXV

SEQ ID NO: 409 - protein, 9 aa, Artificial
  peptide
  misc_feature (8)..(9): Xaa can be any naturally occurring amino acid
VLIDKTSXX

SEQ ID NO: 410 - protein, 9 aa, SEQ ID NO: 411
  misc_feature (2)..(2): Xaa can be any naturally occurring amino acid
VXIDKTSSV

SEQ ID NO: 411 - protein, 9 aa, Artificial
  peptide
  misc_feature (8)..(9): Xaa can be any naturally occurring amino acid
YLIDKTSXX

SEQ ID NO: 412 - protein, 9 aa, Artificial
  peptide
  misc_feature (1)..(1): Xaa can be any naturally occurring amino acid
  misc_feature (8)..(8): Xaa can be any naturally occurring amino acid
XLIDKTSXA

SEQ ID NO: 413 - protein, 9 aa, Artificial
  peptide
  misc_feature (1)..(1): Xaa can be any naturally occurring amino acid
  misc_feature (8)..(8): Xaa can be any naturally occurring amino acid
XLIDKTSXV

SEQ ID NO: 414 - protein, 9 aa, Artificial
  peptide
  misc_feature (1)..(1): Xaa can be any naturally occurring amino acid
  misc_feature (8)..(9): Xaa can be any naturally occurring amino acid
XLIDKTSXX

SEQ ID NO: 415 - protein, 9 aa, Artificial
  peptide
  misc_feature (2)..(2): Xaa can be any naturally occurring amino acid
  misc_feature (8)..(8): Xaa can be any naturally occurring amino acid
FXLLFATXV

SEQ ID NO: 416 - protein, 9 aa, Artificial
  peptide
  misc_feature (8)..(8): Xaa can be any naturally occurring amino acid
LLLLFATXV

SEQ ID NO: 417 - protein, 9 aa, Artificial
  peptide
  misc_feature (2)..(2): Xaa can be any naturally occurring amino acid
  misc_feature (8)..(8): Xaa can be any naturally occurring amino acid
LXLLFATXV

SEQ ID NO: 418 - protein, 9 aa, Artificial
  peptide
  misc_feature (8)..(9): Xaa can be any naturally occurring amino acid
YLLLFATXX

SEQ ID NO: 419 - protein, 9 aa, Artificial
  peptide
  misc_feature (1)..(2): Xaa can be any naturally occurring amino acid
XXLLFATSV

SEQ ID NO: 420 - protein, 9 aa, Artificial
  peptide
  misc_feature (1)..(1): Xaa can be any naturally occurring amino acid
  misc_feature (8)..(9): Xaa can be any naturally occurring amino acid
XMLLFATXX

SEQ ID NO: 421 - protein, 9 aa, Artificial
  peptide
  misc_feature (1)..(2): Xaa can be any naturally occurring amino acid
  misc_feature (8)..(8): Xaa can be any naturally occurring amino acid
XXVGICLXV

SEQ ID NO: 422 - protein, 9 aa, Artificial
  peptide
  misc_feature (8)..(8): Xaa can be any naturally occurring amino acid
KLIKYFLXV

SEQ ID NO: 423 - protein, 9 aa, Artificial
  peptide
  misc_feature (1)..(1): Xaa can be any naturally occurring amino acid
  misc_feature (8)..(8): Xaa can be any naturally occurring amino acid
XLIKYFLXV

SEQ ID NO: 424 - protein, 9 aa, Artificial
  peptide
  misc_feature (1)..(1): Xaa can be any naturally occurring amino acid
  misc_feature (8)..(9): Xaa can be any naturally occurring amino acid
XLIKYFLXX

SEQ ID NO: 425 - protein, 9 aa, Artificial
  peptide
  misc_feature (1)..(2): Xaa can be any naturally occurring amino acid
  misc_feature (8)..(8): Xaa can be any naturally occurring amino acid
XXIKYFLXV

SEQ ID NO: 426 - protein, 9 aa, Artificial
  peptide
  misc_feature (8)..(8): Xaa can be any naturally occurring amino acid
ALVLALVXV

SEQ ID NO: 427 - protein, 9 aa, Artificial
  peptide
  misc_feature (8)..(8): Xaa can be any naturally occurring amino acid
SLVLALVXV

SEQ ID NO: 428 - protein, 9 aa, Artificial
  peptide
  misc_feature (1)..(1): Xaa can be any naturally occurring amino acid
  misc_feature (8)..(8): Xaa can be any naturally occurring amino acid
XLVLALVXV

SEQ ID NO: 429 - protein, 9 aa, Artificial
  peptide
  misc_feature (8)..(8): Xaa can be any naturally occurring amino acid
ALALVLAXL

SEQ ID NO: 430 - protein, 9 aa, Artificial
  peptide
  misc_feature (8)..(9): Xaa can be any naturally occurring amino acid
ALALVLAXX

SEQ ID NO: 431 - protein, 9 aa, Artificial
  peptide
  misc_feature (9)..(9): Xaa can be any naturally occurring amino acid
FLALVLAAX

SEQ ID NO: 432 - protein, 9 aa, Artificial
  peptide
  misc_feature (8)..(8): Xaa can be any naturally occurring amino acid
FLALVLAXL

SEQ ID NO: 433 - protein, 9 aa, Artificial
  peptide
  misc_feature (8)..(8): Xaa can be any naturally occurring amino acid
GLALVLAXI

SEQ ID NO: 434 - protein, 9 aa, Artificial
  peptide
  misc_feature (8)..(8): Xaa can be any naturally occurring amino acid
GLALVLAXL

SEQ ID NO: 435 - protein, 9 aa, Artificial
  peptide
  misc_feature (8)..(8): Xaa can be any naturally occurring amino acid
GLALVLAXV

SEQ ID NO: 436 - protein, 9 aa, Artificial
  peptide
  misc_feature (2)..(2): Xaa can be any naturally occurring amino acid
GXALVLAVV

SEQ ID NO: 437 - protein, 9 aa, Artificial
  peptide
  misc_feature (9)..(9): Xaa can be any naturally occurring amino acid
SLALVLALX

SEQ ID NO: 438 - protein, 9 aa, Artificial
  peptide
  misc_feature (9)..(9): Xaa can be any naturally occurring amino acid
VLALVLAEX

SEQ ID NO: 439 - protein, 9 aa, Artificial
  peptide
  misc_feature (8)..(8): Xaa can be any naturally occurring amino acid
VLALVLAXV

SEQ ID NO: 440 - protein, 9 aa, Artificial
  peptide
  misc_feature (8)..(8): Xaa can be any naturally occurring amino acid
YLALVLAXL

SEQ ID NO: 441 - protein, 9 aa, Artificial
  peptide
  misc_feature (1)..(1): Xaa can be any naturally occurring amino acid
XLALVLAEV

SEQ ID NO: 442 - protein, 9 aa, Artificial
  peptide
  misc_feature (1)..(1): Xaa can be any naturally occurring amino acid
XLALVLALL

SEQ ID NO: 443 - protein, 9 aa, Artificial
  peptide
  misc_feature (1)..(1): Xaa can be any naturally occurring amino acid
XLALVLAML

SEQ ID NO: 444 - protein, 9 aa, Artificial
  peptide
  misc_feature (1)..(1): Xaa can be any naturally occurring amino acid
  misc_feature (8)..(8): Xaa can be any naturally occurring amino acid
XLALVLAXL

SEQ ID NO: 445 - protein, 9 aa, Artificial
  peptide
  misc_feature (1)..(1): Xaa can be any naturally occurring amino acid
  misc_feature (8)..(8): Xaa can be any naturally occurring amino acid
XLALVLAXI

SEQ ID NO: 446 - protein, 9 aa, Artificial
  peptide
  misc_feature (1)..(1): Xaa can be any naturally occurring amino acid
  misc_feature (8)..(8): Xaa can be any naturally occurring amino acid
XLALVLAXV

SEQ ID NO: 447 - protein, 9 aa, Artificial
  peptide
  misc_feature (8)..(9): Xaa can be any naturally occurring amino acid
ALFGAPAXX

SEQ ID NO: 448 - protein, 9 aa, Artificial
  peptide
  misc_feature (8)..(8): Xaa can be any naturally occurring amino acid
LLFGAPAXL

SEQ ID NO: 449 - protein, 9 aa, Artificial
  peptide
  misc_feature (9)..(9): Xaa can be any naturally occurring amino acid
LLFGAPAGX

SEQ ID NO: 450 - protein, 9 aa, Artificial
  peptide
  misc_feature (8)..(8): Xaa can be any naturally occurring amino acid
LMFGAPAXV

SEQ ID NO: 451 - protein, 9 aa, Artificial
  peptide
  misc_feature (8)..(8): Xaa can be any naturally occurring amino acid
VLFGAPAXL

SEQ ID NO: 452 - protein, 9 aa, Artificial
  peptide
  misc_feature (1)..(1): Xaa can be any naturally occurring amino acid
  misc_feature (8)..(8): Xaa can be any naturally occurring amino acid
XLFGAPAXA

SEQ ID NO: 453 - protein, 9 aa, Artificial
  peptide
  misc_feature (1)..(1): Xaa can be any naturally occurring amino acid
  misc_feature (8)..(8): Xaa can be any naturally occurring amino acid
XLFGAPAXI

SEQ ID NO: 454 - protein, 9 aa, Artificial
  peptide
  misc_feature (1)..(1): Xaa can be any naturally occurring amino acid
  misc_feature (8)..(8): Xaa can be any naturally occurring amino acid
XMFGAPAXV

SEQ ID NO: 455 - protein, 9 aa, Artificial
  peptide
  misc_feature (1)..(2): Xaa can be any naturally occurring amino acid
  misc_feature (8)..(8): Xaa can be any naturally occurring amino acid
XXFGAPAXV

SEQ ID NO: 456 - protein, 9 aa, Artificial
  peptide
  misc_feature (2)..(2): Xaa can be any naturally occurring amino acid
  misc_feature (8)..(8): Xaa can be any naturally occurring amino acid
FXPGLLFXV

SEQ ID NO: 457 - protein, 9 aa, Artificial
  peptide
  misc_feature (9)..(9): Xaa can be any naturally occurring amino acid
ILPGLLFYX

SEQ ID NO: 458 - protein, 9 aa, Artificial
  peptide
  misc_feature (8)..(8): Xaa can be any naturally occurring amino acid
ILPGLLFXI

SEQ ID NO: 459 - protein, 9 aa, Artificial
  peptide
  misc_feature (8)..(8): Xaa can be any naturally occurring amino acid
ILPGLLFXL

SEQ ID NO: 460 - protein, 9 aa, Artificial
  peptide
  misc_feature (8)..(9): Xaa can be any naturally occurring amino acid
IMPGLLFXX

SEQ ID NO: 461 - protein, 9 aa, Artificial
  peptide
  misc_feature (8)..(9): Xaa can be any naturally occurring amino acid
KLPGLLFXX

SEQ ID NO: 462 - protein, 9 aa, Artificial
  peptide
  misc_feature (8)..(9): Xaa can be any naturally occurring amino acid
LLPGLLFXX

SEQ ID NO: 463 - protein, 9 aa, Artificial
  peptide
  misc_feature (8)..(9): Xaa can be any naturally occurring amino acid
MLPGLLFXX

SEQ ID NO: 464 - protein, 9 aa, Artificial
  peptide
  misc_feature (8)..(9): Xaa can be any naturally occurring amino acid
SLPGLLFXX

SEQ ID NO: 465 - protein, 9 aa, Artificial
  peptide
  misc_feature (9)..(9): Xaa can be any naturally occurring amino acid
TLPGLLFPX

SEQ ID NO: 466 - protein, 9 aa, Artificial
  peptide
  misc_feature (8)..(8): Xaa can be any naturally occurring amino acid
VLPGLLFXV

SEQ ID NO: 467 - protein, 9 aa, Artificial
  peptide
  misc_feature (1)..(1): Xaa can be any naturally occurring amino acid
  misc_feature (8)..(9): Xaa can be any naturally occurring amino acid
XMPGLLFXX

SEQ ID NO: 468 - protein, 9 aa, Artificial
  peptide
  misc_feature (1)..(1): Xaa can be any naturally occurring amino acid
XLPGLLFSV

SEQ ID NO: 469 - protein, 9 aa, Artificial
  peptide
  misc_feature (1)..(1): Xaa can be any naturally occurring amino acid
XLPGLLFVV

SEQ ID NO: 470 - protein, 9 aa, Artificial
  peptide
  misc_feature (1)..(1): Xaa can be any naturally occurring amino acid
  misc_feature (8)..(8): Xaa can be any naturally occurring amino acid
XLPGLLFXM

SEQ ID NO: 471 - protein, 9 aa, Artificial
  peptide
  misc_feature (1)..(1): Xaa can be any naturally occurring amino acid
  misc_feature (8)..(8): Xaa can be any naturally occurring amino acid
XLPGLLFXL

SEQ ID NO: 472 - protein, 9 aa, Artificial
  peptide
  misc_feature (1)..(1): Xaa can be any naturally occurring amino acid
  misc_feature (8)..(8): Xaa can be any naturally occurring amino acid
XLPGLLFXV

SEQ ID NO: 473 - protein, 20 aa, Artificial
  peptide
MAKTIAYDEEARRGLERGLN

SEQ ID NO: 474 - protein, 13 aa, Artificial
  peptide
TPPAYRPPNAPIL

SEQ ID NO: 475 - protein, 15 aa, Artificial
  peptide
KSVWSKLQSIGIRQH

SEQ ID NO: 476 - protein, 9 aa, Artificial Sequence
  peptide
AMNSLSLLL

SEQ ID NO: 477 - protein, 9 aa, Artificial Sequence
  peptide
AMNSLSLTV

SEQ ID NO: 478 - protein, 9 aa, Artificial Sequence
  peptide
GMNSLSLLV

SEQ ID NO: 479 - protein, 9 aa, Artificial Sequence
  peptide
ILNSLSLDI

SEQ ID NO: 480 - protein, 9 aa, Artificial Sequence
  peptide
ILNSLSLTA

SEQ ID NO: 481 - protein, 9 aa, Artificial Sequence
  peptide
QMNSLSLFL

SEQ ID NO: 482 - protein, 9 aa, Artificial Sequence
  peptide
VLNSLSLYA

SEQ ID NO: 483 - protein, 9 aa, Artificial Sequence
  peptide
VMNSLSLLI

SEQ ID NO: 484 - protein, 9 aa, Artificial Sequence
  peptide
YINSLSLFI

SEQ ID NO: 485 - protein, 9 aa, Artificial Sequence
  peptide
FLFEHPETF

SEQ ID NO: 486 - protein, 9 aa, Artificial Sequence
  peptide
HIFEHPEHL

SEQ ID NO: 487 - protein, 9 aa, Artificial Sequence
  peptide
RVFEHPERV

SEQ ID NO: 488 - protein, 9 aa, Artificial Sequence
  peptide
YTFEHPETI

SEQ ID NO: 489 - protein, 9 aa, Artificial Sequence
  peptide
ALAFVPLWL

SEQ ID NO: 490 - protein, 9 aa, Artificial Sequence
  peptide
AMAFVPLAL

SEQ ID NO: 491 - protein, 9 aa, Artificial Sequence
  peptide
FLAFVPLDV

SEQ ID NO: 492 - protein, 9 aa, Artificial Sequence
  peptide
LLAFVPLPL

SEQ ID NO: 493 - protein, 9 aa, Artificial Sequence
  peptide
VLAFVPLGV

SEQ ID NO: 494 - protein, 9 aa, Artificial Sequence
  peptide
ALFGAPAAA

SEQ ID NO: 495 - protein, 9 aa, Artificial Sequence
  peptide
ILFGAPAGA

SEQ ID NO: 496 - protein, 9 aa, Artificial Sequence
  peptide
NMFGAPAQV

SEQ ID NO: 497 - protein, 9 aa, Artificial Sequence
  peptide
SLFGAPATA

SEQ ID NO: 498 - protein, 9 aa, Artificial Sequence
  peptide
TLFGAPAAA

SEQ ID NO: 499 - protein, 9 aa, Artificial Sequence
  peptide
VIFGAPALV

SEQ ID NO: 500 - protein, 9 aa, Artificial Sequence
  peptide
VLFGAPAGI

SEQ ID NO: 501 - protein, 9 aa, Artificial Sequence
  peptide
  MISC_FEATURE (8)..(9): Xaa can be any naturally occurring amino acid
AMNSLSLXX

SEQ ID NO: 502 - protein, 9 aa, Artificial Sequence
  peptide
  MISC_FEATURE (1)..(1): Xaa can be any naturally occurring amino acid
  MISC_FEATURE (9)..(9): Xaa can be any naturally occurring amino acid
XMNSLSLLX

SEQ ID NO: 503 - protein, 9 aa, Artificial Sequence
  peptide
  MISC_FEATURE (1)..(1): Xaa can be any naturally occurring amino acid
  MISC_FEATURE (8)..(8): Xaa can be any naturally occurring amino acid
XMNSLSLXI

SEQ ID NO: 504 - protein, 9 aa, Artificial Sequence
  peptide
  MISC_FEATURE (1)..(1): Xaa can be any naturally occurring amino acid
  MISC_FEATURE (8)..(8): Xaa can be any naturally occurring amino acid
XMNSLSLXL

SEQ ID NO: 505 - protein, 9 aa, Artificial Sequence
  peptide
  MISC_FEATURE (2)..(2): Xaa can be any naturally occurring amino acid
  MISC_FEATURE (9)..(9): Xaa can be any naturally occurring amino acid
YXFEHPETX

SEQ ID NO: 506 - protein, 9 aa, Artificial Sequence
  peptide
  MISC_FEATURE (9)..(9): Xaa can be any naturally occurring amino acid
ALFGAPAAX

SEQ ID NO: 507 - protein, 9 aa, Artificial Sequence
  peptide
  MISC_FEATURE (8)..(9): Xaa can be any naturally occurring amino acid
VLFGAPAXX

SEQ ID NO: 508 - protein, 9 aa, Artificial Sequence
  peptide
  MISC_FEATURE (1)..(1): Xaa can be any naturally occurring amino acid
XLFGAPAAA

SEQ ID NO: 509 - protein, 9 aa, Artificial Sequence
  peptide
  MISC_FEATURE (1)..(1): Xaa can be any naturally occurring amino acid
XMFGAPALV